European Patent Specification EP 4 085 156 B1, published October 25, 2023. Title: QUANTITATIVE PCR SCREENING OF INDUCIBLE PROPHAGE FROM BACTERIAL ISOLATES. Applicant: F. Hoffmann-La Roche AG Roche Diagnostics GmbH Roche Molecular Systems, Inc. The sequence listing filed with the application follows.

SEQUENCE LISTING (99 sequences)

SEQ ID NO: 1 - DNA, 25 bp, Artificial Sequence
  Klebsiella pneumoniae Clade 01 primer1
gggctatcacatatcacgtttgtac

SEQ ID NO: 2 - DNA, 18 bp, Artificial Sequence
  Klebsiella pneumoniae Clade 02 primer1
tgcaaggtggtggtgacc

SEQ ID NO: 3 - DNA, 20 bp, Artificial Sequence
  Klebsiella pneumoniae Clade 03 primer1
atgaagcctgagcatctcaa

SEQ ID NO: 4 - DNA, 16 bp, Artificial Sequence
  Klebsiella pneumoniae Clade 04 primer1
actccgtcccgtggga

SEQ ID NO: 5 - DNA, 23 bp, Artificial Sequence
  Klebsiella pneumoniae Clade 05 primer1
gacaatttgtcggtcgatggaaa

SEQ ID NO: 6 - DNA, 23 bp, Artificial Sequence
  Klebsiella pneumoniae Clade 06 primer1
gcctgaatatgtcatccaccaac

SEQ ID NO: 7 - DNA, 14 bp, Artificial Sequence
  Klebsiella pneumoniae Clade 07 primer1
cgccgggatccgga

SEQ ID NO: 8 - DNA, 20 bp, Artificial Sequence
  Klebsiella pneumoniae Clade 08 primer1
ggcgaaattccggcctgtaa

SEQ ID NO: 9 - DNA, 19 bp, Artificial Sequence
  Klebsiella pneumoniae Clade 09 primer1
tgctggtggagttctggac

SEQ ID NO: 10 - DNA, 20 bp, Artificial Sequence
  Klebsiella pneumoniae Clade 10 primer1
ggcaacctatccgaacgtca

SEQ ID NO: 11 - DNA, 22 bp, Artificial Sequence
  Klebsiella pneumoniae Clade 11 primer1
actacgatgatttgcgtgggtc

SEQ ID NO: 12 - DNA, 22 bp, Artificial Sequence
  Klebsiella pneumoniae Clade 12 primer1
tggtatctggcgatatcgttgc

SEQ ID NO: 13 - DNA, 29 bp, Artificial Sequence
  Klebsiella pneumoniae Clade 01 primer2
acaaaacgcatatggtcaaagttcttaaa

SEQ ID NO: 14 - DNA, 20 bp, Artificial Sequence
  Klebsiella pneumoniae Clade 02 primer2
ggatcgttgctgtacatcgc

SEQ ID NO: 15 - DNA, 26 bp, Artificial Sequence
  Klebsiella pneumoniae Clade 03 primer2
tgtcggtgatccagtaaagattgttc

SEQ ID NO: 16 - DNA, 24 bp, Artificial Sequence
  Klebsiella pneumoniae Clade 04 primer2
tgtagacaatccagccatcaatca

SEQ ID NO: 17 - DNA, 21 bp, Artificial Sequence
  Klebsiella pneumoniae Clade 05 primer2
cgcgattatttttcgccacgc

SEQ ID NO: 18 - DNA, 24 bp, Artificial Sequence
  Klebsiella pneumoniae Clade 06 primer2
gacaccgtcgatttgaatctcttc

SEQ ID NO: 19 - DNA, 27 bp, Artificial Sequence
  Klebsiella pneumoniae Clade 07 primer2
cgaaattaaggactttgtgggcatcaa

SEQ ID NO: 20 - DNA, 21 bp, Artificial Sequence
  Klebsiella pneumoniae Clade 08 primer2
ggagaacgcaataaaccgctc

SEQ ID NO: 21 - DNA, 23 bp, Artificial Sequence
  Klebsiella pneumoniae Clade 09 primer2
gcaacaaagccatatttcaccgc

SEQ ID NO: 22 - DNA, 20 bp, Artificial Sequence
  Klebsiella pneumoniae Clade 10 primer2
atgtcgctgacaggcaagta

SEQ ID NO: 23 - DNA, 20 bp, Artificial Sequence
  Klebsiella pneumoniae Clade 11 primer2
accgacaagtcgacagcatc

SEQ ID NO: 24 - DNA, 23 bp, Artificial Sequence
  Klebsiella pneumoniae Clade 12 primer2
cgcggccttcatcaaaataaaca

SEQ ID NO: 25 - DNA, 21 bp, Artificial Sequence
  Enterobacter cloacae Clade 02 primer1
cgggaagatatgcgccaagta

SEQ ID NO: 26 - DNA, 18 bp, Artificial Sequence
  Enterobacter cloacae Clade 03 primer1
ggaagagcagctcgtcga

SEQ ID NO: 27 - DNA, 19 bp, Artificial Sequence
  Enterobacter cloacae Clade 04 primer1
gggatcagcccgacactta

SEQ ID NO: 28 - DNA, 19 bp, Artificial Sequence
  Enterobacter cloacae Clade 05 primer2
tgcaggaggtgaaacaggc

SEQ ID NO: 29 - DNA, 19 bp, Artificial Sequence
  Enterobacter cloacae Clade 06 primer1
tgcgcagttagccaggttc

SEQ ID NO: 30 - DNA, 16 bp, Artificial Sequence
  Enterobacter cloacae Clade 07 primer1
cctgccctgactgggc

SEQ ID NO: 31 - DNA, 20 bp, Artificial Sequence
  Enterobacter cloacae Clade 08 primer1
gatggcatggtcgcaatgac

SEQ ID NO: 32 - DNA, 21 bp, Artificial Sequence
  Enterobacter cloacae Clade 09 primer1
acagtcacgacaatgacgaca

SEQ ID NO: 33 - DNA, 21 bp, Artificial Sequence
  Enterobacter cloacae Clade 10 primer1
ggcgattttgttcgccatcac

SEQ ID NO: 34 - DNA, 19 bp, Artificial Sequence
  Enterobacter cloacae Clade 11 primer1
ttgcagaaggcatccgcta

SEQ ID NO: 35 - DNA, 24 bp, Artificial Sequence
  Enterobacter cloacae Clade 02 primer2
tggcagtaatcgaagaagtaaccc

SEQ ID NO: 36 - DNA, 17 bp, Artificial Sequence
  Enterobacter cloacae Clade 03 primer2
gccagctctgtgccctc

SEQ ID NO: 37 - DNA, 17 bp, Artificial Sequence
  Enterobacter cloacae Clade 04 primer2
cgccacaacccacccac

SEQ ID NO: 38 - DNA, 19 bp, Artificial Sequence
  Enterobacter cloacae Clade 05 primer2
cgaggttatgccgcagacc

SEQ ID NO: 39 - DNA, 18 bp, Artificial Sequence
  Enterobacter cloacae Clade 06 primer2
ccgtcgttgaacaggcga

SEQ ID NO: 40 - DNA, 24 bp, Artificial Sequence
  Enterobacter cloacae Clade 07 primer2
atcaacgattttcagttgcctgaa

SEQ ID NO: 41 - DNA, 21 bp, Artificial Sequence
  Enterobacter cloacae Clade 08 primer2
cagcggtcggaaaatgaagtc

SEQ ID NO: 42 - DNA, 20 bp, Artificial Sequence
  Enterobacter cloacae Clade 09 primer2
tgagttggctcgggtcgata

SEQ ID NO: 43 - DNA, 18 bp, Artificial Sequence
  Enterobacter cloacae Clade 10 primer2
acctcgctttcgtcgtcc

SEQ ID NO: 44 - DNA, 22 bp, Artificial Sequence
  Enterobacter cloacae Clade 11 primer2
cactgaagaaaataccgcgctc

SEQ ID NO: 45 - DNA, 19 bp, Artificial Sequence
  Escherichia coli Clade M01 primer1
cgggagtaccgtaaagccc

SEQ ID NO: 46 - DNA, 20 bp, Artificial Sequence
  Escherichia coli Clade M02 primer1
ccgatttatccggaccaggc

SEQ ID NO: 47 - DNA, 16 bp, Artificial Sequence
  Escherichia coli Clade M03 primer1
accaggccgcacatgc

SEQ ID NO: 48 - DNA, 16 bp, Artificial Sequence
  Escherichia coli Clade M04 primer1
ggagccgttcccgcaa

SEQ ID NO: 49 - DNA, 26 bp, Artificial Sequence
  Escherichia coli Clade M05 primer1
ctgtattgttttgcctgtgataacga

SEQ ID NO: 50 - DNA, 14 bp, Artificial Sequence
  Escherichia coli Clade M06 primer1
cgcgccgggcttga

SEQ ID NO: 51 - DNA, 17 bp, Artificial Sequence
  Escherichia coli Clade M07 primer1
ccggtccgtgggagtca

SEQ ID NO: 52 - DNA, 19 bp, Artificial Sequence
  Escherichia coli Clade M08 primer1
tcaggaaaccgcaaaggca

SEQ ID NO: 53 - DNA, 15 bp, Artificial Sequence
  Escherichia coli Clade M09 primer1
cgcgtcagcccggaa

SEQ ID NO: 54 - DNA, 18 bp, Artificial Sequence
  Escherichia coli Clade M10 primer1
gccagcatggagcaacga

SEQ ID NO: 55 - DNA, 23 bp, Artificial Sequence
  Escherichia coli Clade M11 primer1
tgcttgatggtcgcttcaaagta

SEQ ID NO: 56 - DNA, 18 bp, Artificial Sequence
  Escherichia coli Clade M12 primer1
gctgttccgggtgatccc

SEQ ID NO: 57 - DNA, 22 bp, Artificial Sequence
  Escherichia coli Clade M13 primer1
cgcagattcagcgcaaattcaa

SEQ ID NO: 58 - DNA, 24 bp, Artificial Sequence
  Escherichia coli Clade M14 primer1
gcaggaaaaaaatactgtgggaca

SEQ ID NO: 59 - DNA, 18 bp, Artificial Sequence
  Escherichia coli Clade M15 primer1
ctggacggcgtacagtcc

SEQ ID NO: 60 - DNA, 18 bp, Artificial Sequence
  Escherichia coli Clade M16 primer1
agacagaggcgcagcaac

SEQ ID NO: 61 - DNA, 22 bp, Artificial Sequence
  Escherichia coli Clade M17 primer1
actaccgtgaaaaatccgtgga

SEQ ID NO: 62 - DNA, 20 bp, Artificial Sequence
  Escherichia coli Clade M18 primer1
gctgcgcatcagtatttccc

SEQ ID NO: 63 - DNA, 20 bp, Artificial Sequence
  Escherichia coli Clade M01 primer2
ccctgctgctcccagaaatc

SEQ ID NO: 64 - DNA, 18 bp, Artificial Sequence
  Escherichia coli Clade M02 primer2
ccgccaccaggtcaaaca

SEQ ID NO: 65 - DNA, 19 bp, Artificial Sequence
  Escherichia coli Clade M03 primer2
ccaccaggtcaaacaccca

SEQ ID NO: 66 - DNA, 19 bp, Artificial Sequence
  Escherichia coli Clade M04 primer2
tcgcgtcactctgcatcac

SEQ ID NO: 67 - DNA, 20 bp, Artificial Sequence
  Escherichia coli Clade M05 primer2
acctcaatcccgaacgcttc

SEQ ID NO: 68 - DNA, 20 bp, Artificial Sequence
  Escherichia coli Clade M06 primer2
gcgcctcgcgggaaaaataa

SEQ ID NO: 69 - DNA, 19 bp, Artificial Sequence
  Escherichia coli Clade M07 primer2
tgccgtacacaatccagcc

SEQ ID NO: 70 - DNA, 17 bp, Artificial Sequence
  Escherichia coli Clade M08 primer2
gccaccagcggatccca

SEQ ID NO: 71 - DNA, 20 bp, Artificial Sequence
  Escherichia coli Clade M09 primer2
ggccagccgattttcaggta

SEQ ID NO: 72 - DNA, 20 bp, Artificial Sequence
  Escherichia coli Clade M10 primer2
cctgaaccacaaaacggcga

SEQ ID NO: 73 - DNA, 22 bp, Artificial Sequence
  Escherichia coli Clade M11 primer2
cgcatcatgtatgcatagcgaa

SEQ ID NO: 74 - DNA, 25 bp, Artificial Sequence
  Escherichia coli Clade M12 primer2
ccgtaccgatttcggtaaggtaaac

SEQ ID NO: 75 - DNA, 21 bp, Artificial Sequence
  Escherichia coli Clade M13 primer2
cgcatcagccaggttaggaga

SEQ ID NO: 76 - DNA, 20 bp, Artificial Sequence
  Escherichia coli Clade M14 primer2
ctgccagcgggaaatactga

SEQ ID NO: 77 - DNA, 19 bp, Artificial Sequence
  Escherichia coli Clade M15 primer2
cccagcgtggtgttcacaa

SEQ ID NO: 78 - DNA, 20 bp, Artificial Sequence
  Escherichia coli Clade M16 primer2
gcacggacacacgtaatgcc

SEQ ID NO: 79 - DNA, 27 bp, Artificial Sequence
  Escherichia coli Clade M17 primer2
ccatacagagccctcaatacgtttatc

SEQ ID NO: 80 - DNA, 23 bp, Artificial Sequence
  Escherichia coli Clade M18 primer2
cattcatcctctccggataaggc

SEQ ID NO: 81 - DNA, 8439 bp, Artificial Sequence
  pZX023 Kpn packaging cell line plasmid
gaagatcctttgatcttttctacggggtctgacgctcagtggaacgaaaactcacgttaagggattttggtcatgagattatcctcgtcaggtggcacttttcggggaaatgtgcgcggaacccctatttgtttatttttctaaatacattcaaatatgtatccgctcatgagacaataaccctgataaatgcttcaataatattgaaaaaggaagagtcgatcgatgaagtttggaaatatttgtttttcgtatcaaccaccaggtgaaactcataagcaagtaatggatcgctttgttcggcttggtatcgcctcagaagaggtagggtttgatacatattggaccttagaacatcattttacagagtttggtcttacgggaaatttatttgttgctgcggctaacctgttaggaagaactaaaacattaaatgttggcactatgggggttgttattccgacagcacacccagttcgacagttagaagacgttttattattagatcaaatgtcgaaaggtcgttttaattttggaaccgttcgagggctataccataaagattttcgagtatttggtgttgatatggaagagtctcgagcaattactcaaaatttctaccagatgataatggaaagcttacagacaggaaccattagctctgatagtgattacattcaatttcctaaggttgatgtatatcccaaagtgtactcaaaaaatgtaccaacccgtatgactgctgagtccgcaagtacgacagaatggctagcaatacaagggctaccaatggttcttagttggattattggtactaatgaaaaaaaagcacagatggaactctataatgaaattgcgacagaatatggtcatgatatatctaaaatagatcattgtatgacttatatttgttctgttgatgatgatgcacaaaaggcgcaagatgtttgtcgggagtttctgaaaaattggtatgactcatatgtaaatgcgaccaatatctttaatgatagcgatcaaactcgtggttatgattatcataaaggtcaatggcgtgattttgttttacaaggacatacaaacaccaatcgacgtgttgattatagcaatggtattaaccccgtaggcactcctgagcagtgtattgaaatcattcaacgtgatattgatgcaacgggtattacaaacattacatgcggatttgaagctaatggaactgaagatgaaataattgcttccatgcgacgctttatgacacaagtcgctcctttcttaaaagaacctaaataaattacttatttgatactagagataataaggaacaagttatgaaatttggattattttttctaaactttcagaaagatggaataacatctgaagaaacgttggataatatggtaaagactgtcacgttaattgattcaactaaatatcattttaatactgcctttgttaatgaacatcacttttcaaaaaatggtattgttggagcacctattaccgcagctggttttttattagggttaacaaataaattacatattggttcattaaatcaagtaattaccacccatcaccctgtacgtgtagcagaagaagccagtttattagatcaaatgtcagagggacgcttcattcttggttttagtgactgcgaaagtgatttcgaaatggaattttttagacgtcatatctcatcaaggcaacaacaatttgaagcatgctatgaaataattaatgacgcattaactacaggttattgccatccccaaaacgacttttatgattttccaaaggtttcaattaatccacactgttacagtgagaatggacctaagcaatatgtatccgctacatcaaaagaagtcgtcatgtgggcagcgaaaaaggcactgcctttaacgtttaagtgggaggataatttagaaaccaaagaacgctatgcaattctatataataaaacagcacaacaatatggtattgatatttcggatgttgatcatcaattaactgtaattgcgaacttaaatgctgatagaagtacggctcaagaagaagtgagagaatacttaaaagactatatcactgaaacttaccctcaaatggacagagatgaaaaaattaactgcattattgaagagaatgcagttgggtctcatgatgactattatgaatcgacaaaattagcagtggaaaaaacagggtctaaaaatattttattatcctttgaatcaatgtccgatattaaagatgtaaaagatattattgatatgttgaaccaaaaaatcgaaatgaatttaccataaggatcctaaaattaaaggcaatttctatattagattgcctttttggcgcgcctattctaatgcataataaatactgataacatcttatattttgtattatattttgtattatcgttgacatgtataattttgatatcaaaaactgattttccctctattattttcgagatttattttcttaattctctttaacaaactagaaatattgtatatacaaaaaattataaataatagatgaatagtttaattataggtgttcatcaatcgaaaaagcaacgtatcttatttaaagtgcgttgcttttttctcatttataaggttaaataattctcatatatcaagcaaagtgacagagctcggtactctcggcttgaacgaattggcggccgccctgcaggatagctgacgaccttaaggataaatttctggtaaggaggacacgtatggaagtgggcaagttggggaagccgtatccgttgctgaatctggcatatgtgggagtataagacgcgcagcgtcgcatcaggcatttttttctgcgccaatgccggtagatagcaatccggcccgaggggcacaaaaaacccctcaagacccgtttagaggccccaaggggttatgctacgatactcaggcgccgggggcggtgtccggcggcccccagaggaactgcgccagttcctccggatcggtgaagccggagagatccagcggggtctcctcgaacacctcgaagtcgtgcaggaaggtgaaggcgagcagttcgcgggcgaagtcctcggtccgcttccactgcgccccgtcgagcagcgcggccaggatctcgcggtcgccccggaaggcgttgagatgcagttgcaccaggctgtagcgggggtctcccgcatagacgtcggtgaagtcgacgatcccggtgacctcggtcgcggccaggtccacgaagatgttggtcccgtgcaggtcgccgtggacgaaccggggttcgcggccggccagcagcgtgtccacgtccggcagccagtcctccaggcggtccagcagccggggcgagaggtagccccacccgcggtggtcctcgacggtcgccgcgcggcgttcccgcagcagttccgggaagacctcggaatggggggtgagcacggtgttcccggtcagcggcaccctgtgcagccggccgagcacccggccgagttcgcgggccagggcgagcagcgcgttccggtcggtcgtgccgtccatcgcggaccgccaggtggtgccggtcacccggctcatcaccaggtagggccacggccaggctccggtgccgggccgcagctcgccgcggccgaggaggcggggcaccggcaccggggcgtccgccaggaccgcgtacgcctccgactccgacgcgaggctctccggaccgcaccagtgctcgccgaacagcttgatcaccgggccgggctcgccgaccagtacggggttggtgctctcgccgggcacccgcagcaccggcggcaccggcagcccgagctcctccagggctcggcgggccagcggctcccagaattcctggtcgttccgcaggctcgcgtaggaatcatccgaatcaatacggtcgagaagtaacagggattcttgtgtcatatgaatcttactcctttgttaaattatttttgtttaagcattttgaatttgtatgcatcttagaacaatctcaaagttccaagctcttgcaagtctagatattgagtcaaaaaaaattttcaactcatactcttcctttttcaatattattgaagcatttatcagggttattgtctcatgagcgcacatttccccgaaaagtgccacctgacgtctaagaaaccattattatcatgacattaacctataaaaataggcgtatcacgaggccctttcgtctcgcgcgtttcggtgatgacggtgaaaacctctgacacatgcagctcccggagacggtcacagcttgtctgtaagcggatgccgggagcagacaagcccgtcagggcgcgtcagcgggtgttggcgggtgtcggggctggcttaactatgcggcatcagagcagattgtactgagagtgcaccatatgcggtgtgaaataccgcacagatgcgtaaggagaaaataccgcatcaggcgccattcgccattcaggctgcgcaactgttgggaagggcgatcggtgcgggcctcttcgctattacgccagctggcgaaagggggatgtgctgcaaggcgattaagttgggtaacgccagggttttcccagtcacgacgttgtaaaacgacggccagtgaattcgagctcggtacccggggatcctctagagtcgacctgcaggcatgcaagcttggcgtaatcatggtcatagctgtttcctgtgtgaaattgttatccgctcacaattccacacaacatacgagccggaagcataaagtgtaaagcctggggtgcctaatgagtgagctcagcaggcattacaacaggcgctcacagagcgcctgtgataatggctgaatgcttcaccagcgcggcgttttatgggaggtcatgatgagttacaccagctgtacttattgcggttcacgtctccatacgcgggctaactgcccgaaaacatggggcggttcatcgcgtcgcgccaatctgcgctgcagctattgtggccagtccgggcataactcgaatgcctgcccacataatgcgagcagcagtcggcggcgcagcctgaatgacgacttccacctcgactgaggcagccgccgtcatggggtaggggggatcaaatccctaacccctttcgcgcttcgggactgccgcttcaggtagatttttgcgcgtgagaaataaaaactttttttttggctgttttggggtgcttttgaatgagtacagggatgcgatcacctggtggcggacgcaaatcgaataacactggaaatcaggttagttctttaaccagagcggtttctccgccggatgaattactgggcgatatggctatcgatgcctggaaacggacgtgcaaaattcttattaaccgtggcacgttcgaaatggaagattgttatttgctgatggaatactgcaacaccgtgcagctgctgtacgacgccaaccaggaaattaaaagcgatggccttggtgatgataccgctgccggcggtcagaaacttggtgcggcagtgaaggcgcgtagccgttatatcagcgaattaattcgactctccgttgtgttaaagctggaccccaatagccgcatcctgaagaaacagcccggagataatgacaaatccagcggtgagttcgacgagttttaattttggtgcggccctaatgacttaaggatggagcatggccgcatatccaaacgtcaatgtggcgaacaaatatgcgcgggatatcatagacgggaaaatagtcgcctgcagagctattcggctggcatgtcagcgccattttgacgatttaaaaaaatcactcgataacaataacccttaccggttcgacagagatttagctgagcgggcctgccggtttgttcagaagttaccgcactccagtggcgatttggcgggacagaaattaaaactggaaccttggcaaagttttattttttgttcgatttttggctgggtcacgaaaaaggataaaaaacgccgatttcgcgaagcgtatatccgggtagctaggaaaaacgggaaatcgttttttgctgccgggattggcacctacatgttttgcgctgatggcgaaaacagtgcagaagtgtattgcggtgcgacaactatggcgcaggcgaaaaaggtcttcaccccagccaggcagatggccagccgcctgccggcacttcgctccagatttgatatttcggtatggaccgacagcctgacacgcccggatggttccgttttcgcacctatggcggggaaacccggcgatggtgacagcccacattgcgcgatcattgacgagtatcacgaacacgatacggatcatatgtacgaggccatgacaatggggatgggcgcccgttcgcagccgttaacgctcattatcacgacagccggctcgtcactggagtcaccttgctatgacaaggacaaggaagtcaaagaggttatcgaaggcataacccgtaatgatcgcctgtttggcatgatttacgaactggatgctggcgatgactggaccgacccgaaaaacttaatcaaagctaacccaaatctggacgtttcggttaagtacagcgacctggttgagcttctggaagtagcgaaacaggttcctcgcaaggttaacgccttcaaaaccaaacgcctcaatatttgggtatccggtaaatccgcgttctacaacatggagcagtggaaggctgctgaagaccccgaccttgagctggctgattttgcgaatgacagctgcaacatcggtctcgatctcgccaaaaagctggatatgaacgccgggatacggctatttacgcgggaaattgaaggtaaacggcattattactgcatcaaacctaaattttgggtcccggaagacactatccatacaaccgatccaaaactgctgaaaactgctgacaggtatcagaagttttatgaaatgggcgtgctggaagcgacggatggcgcagaggcagactatcgcgagattctggccagtattatcgatatgcaggacgaaaaccgcattgacgagattgatatcgaccctgccggcgcaacagcacttcgccaccagttggaggacaacggatttaccgtagtcgatatccggcaggattacaccaatatgtcaccggcgatgaaagagcttgaagcggctctggccggtggtcgattccaccatgatggcaatcccattctgacctggtgtatcagcaacgttatcgggaaatttatacccggtagcgatgatctcgttcgcccgacaaagggagacaatcaaagcaaaatcgatggagctacagcgttatttaacgccatgactcgcgcaatgctgcacgaaagcagcggcggcacatcggtatatgatgaggaagacatagcgtgttaatcacaattctgagtttcattattggcctggccggggctgtactcatatccgccggagcctggttgattttgcctgctgccggtcttattacgggcgggtcaatatgtcttatctggtcatatctgactgcgcgggcggtttcagccggtgccaaatttaacgggggtgaataactcacattaattgcgttgcgctcactgcccgctttccagtcgggaaacctgtcgtgccagctgcattaatgaatcggccaacgcgcggggagaggcggtttgcgtattgggcgctcttccgcttcctcgctcactgactcgctgcgctcggtcgttcggctgcggcgagcggtatcagctcactcaaaggcggtaatacggttatccacagaatcaggggataacgcaggaaagaacatgtgagcaaaaggccagcaaaaggccaggaaccgtaaaaaggccgcgttgctggcgtttttccataggctccgcccccctgacgagcatcacaaaaatcgacgctcaagtcagaggtggcgaaacccgacaggactataaagataccaggcgtttccccctggaagctccctcgtgcgctctcctgttccgaccctgccgcttaccggatacctgtccgcctttctcccttcgggaagcgtggcgctttctcatagctcacgctgtaggtatctcagttcggtgtaggtcgttcgctccaagctgggctgtgtgcacgaaccccccgttcagcccgaccgctgcgccttatccggtaactatcgtcttgagtccaacccggtaagacacgacttatcgccactggcagcagccactggtaacaggattagcagagcgaggtatgtaggcggtgctacagagttcttgaagtggtggcctaactacggctacactagaagaacagtatttggtatctgcgctctgctgaagccagttaccttcggaaaaagagttggtagctcttgatccggcaaacaaaccaccgctggtagcggtggtttttttgtttgcaagcagcagattacgcgcagaaaaaaaggatctcaa

SEQ ID NO: 82 - DNA, 20 bp, Artificial Sequence
  Pae060_F10_terL forward primer
acgactgccattggatgtgt

SEQ ID NO: 83 - DNA, 20 bp, Artificial Sequence
  Pae060_F10 terL reverse primer
tgctgtacacccttgacgac

SEQ ID NO: 84 - DNA, 20 bp, Artificial Sequence
  Pae065_F10 terL forward primer
tccaagctgacctatgcacg

SEQ ID NO: 85 - DNA, 20 bp, Artificial Sequence
  Pae065_F10 terL reverse primer
gatccaccgagtagcccatg

SEQ ID NO: 86 - DNA, 20 bp, Artificial Sequence
  Pae042_phi297 terL forward pirmer
gcgactgatcatcaacgtgc

SEQ ID NO: 87 - DNA, 20 bp, Artificial Sequence
  Pae042_phi297 terL reverse primer
cctgatacgccgaggacttc

SEQ ID NO: 88 - DNA, 20 bp, Artificial Sequence
  Pae057_phi3 terL forward primer
atatcctgaagtcgcgccag

SEQ ID NO: 89 - DNA, 20 bp, Artificial Sequence
  Pae057_phi3 terL reverse primer
ttgccggacagctcgatatc

SEQ ID NO: 90 - DNA, 20 bp, Artificial Sequence
  Cfi16709_P1 TF forward primer
cggtgcgactgagatcactt

SEQ ID NO: 91 - DNA, 20 bp, Artificial Sequence
  Cfi16709_P1 TF reverse primer
actgcgaatgtggatcagct

SEQ ID NO: 92 - DNA, 20 bp, Artificial Sequence
  Cfi16710_phiKO2 TF forward primer
cggtatatgaccccacggtg

SEQ ID NO: 93 - DNA, 20 bp, Artificial Sequence
  Cfi16710_phiKO2 TF reverse primer
ggttcacggcccggatatag

SEQ ID NO: 94 - DNA, 20 bp, Artificial Sequence
  Sms16017_SEN34 TF forward primer
cgacgagctgcatgttgatg

SEQ ID NO: 95 - DNA, 20 bp, Artificial Sequence
  Sms16017_SEN34 TF reverse primer
ggtcacatctcgaagcgtca

SEQ ID NO: 96 - DNA, 20 bp, Artificial Sequence
  Sms16926_Psp3 TF forward primer
ccttgctggcaaagggtttc

SEQ ID NO: 97 - DNA, 20 bp, Artificial Sequence
  Sms16926_Psp3 TF reverse primer
cagtacccagctccaggttg

SEQ ID NO: 98 - DNA, 20 bp, Artificial Sequence
  luxA_qPCR forward primer
tgctgcggctaacctgttag

SEQ ID NO: 99 - DNA, 20 bp, Artificial Sequence
  luxA_qPCR reverse primer
tggtatagccctcgaacggt